European Patent Specification EP 4 110 297 B1, published September 3, 2025. Title: CELL-TARGETED NANOPARTICLES TO INHIBIT RNA CARGO. Applicant: THE TRUSTEES OF INDIANA UNIVERSITY SEN, CHANDAN GHATAK, SUBHADIP ROY, SASHWATI. The sequence listing filed with the application follows.

SEQUENCE LISTING (9 sequences)

SEQ ID NO: 1 - protein, 11 aa, Homo sapiens
ASKAIQFLLAG

SEQ ID NO: 2 - RNA, 22 nt, Homo sapiens
ucguaccgugaguaauaaugcg

SEQ ID NO: 3 - RNA, 23 nt, Homo sapiens
guucagaguucuaggagucuuuu

SEQ ID NO: 4 - RNA, 23 nt, Homo sapiens
cacuccuagaacucugaacuuuu

SEQ ID NO: 5 - protein, 12 aa, Homo sapiens
ASKAIQVFLLAG

SEQ ID NO: 6 - RNA, 19 nt, Mus musculus
ggaucugauggauacggaa

SEQ ID NO: 7 - RNA, 19 nt, Mus musculus
gggauggcuauaaugggua

SEQ ID NO: 8 - RNA, 19 nt, Mus musculus
accgauaggcagucuggaa

SEQ ID NO: 9 - RNA, 19 nt, Mus musculus
gguggaauuaaggaagaua